European Patent Specification EP 4 514 813 B1, published August 5, 2026. Title: PSEUDO-DISACCHARIDE COMPOUNDS. Applicant: Universiteit Leiden. Application NL PCT/NL2023/050231, filed April 28, 2023. The sequence listing filed with the application follows.

SEQUENCE LISTING (5 sequences)

SEQ ID NO: 1 - protein, 651 aa, Homo sapiens
MARGSAVAWAALGPLLWGCALGLQGGMLYPQESPSRECKELDGLWSFRADFSDNRRRGFEEQWYRRPLWESGPTVDMPVPSSFNDISQDWRLRHFVGWVWYEREVILPERWTQDLRTRVVLRIGSAHSYAIVWVNGVDTLEHEGGYLPFEADISNLVQVGPLPSRLRITIAINNTLTPTTLPPGTIQYLTDTSKYPKGYFVQNTYFDFFNYAGLQRSVLLYTTPTTYIDDITVITSVEQDSGLVNYQISVKGSNLFKLEVRLLDAENKVVANGTGTQGQLKVPGVSLWWPYLMHERPAYLYSLEVQLTAQTSLGPVSDFYTLPVGIRTVAVTKSQFLINGKPFYFHGVNKHEDADIRGKGFDWPLLVKDFNLLRWLGANAFRTSHYPYAEEVMQMCDRYGIVVIDECPGVGLALPQFFNNVSLHHHMQVMEEVVRRDKNHPAVVMWSVANEPASHLESAGYYLKMVIAHTKSLDPSRPVTFVSNSNYAADKGAPYVDVICLNSYYSWYHDYGHLELIQLQLATQFENWYKKYQKPIIQSEYGAETIAGFHQDPPLMFTEEYQKSLLEQYHLGLDQKRRKYVVGELIWNFADFMTEQSPTRVLGNKKGIFTRQRQPKSAAFLLRERYWKIANETRYPHSVAKSQCLENSLFT

SEQ ID NO: 2 - protein, 603 aa, Escherichia coli
MLRPVETPTREIKKLDGLWAFSLDRENCGIDQRWWESALQESRAIAVPGSFNDQFADADIRNYAGNVWYQREVFIPKGWAGQRIVLRFDAVTHYGKVWVNNQEVMEHQGGYTPFEADVTPYVIAGKSVRITVCVNNELNWQTIPPGMVITDENGKKKQSYFHDFFNYAGIHRSVMLYTTPNTWVDDITVVTHVAQDCNHASVDWQVVANGDVSVELRDADQQVVATGQGTSGTLQVVNPHLWQPGEGYLYELCVTAKSQTECDIYPLRVGIRSVAVKGEQFLINHKPFYFTGFGRHEDADLRGKGFDNVLMVHDHALMDWIGANSYRTSHYPYAEEMLDWADEHGIVVIDETAAVGFNLSLGIGFEAGNKPKELYSEEAVNGETQQAHLQAIKELIARDKNHPSVVMWSIANEPDTRPQGAREYFAPLAEATRKLDPTRPITCVNVMFCDAHTDTISDLFDVLCLNRYYGWYVQSGDLETAEKVLEKELLAWQEKLHQPIIITEYGVDTLAGLHSMYTDMWSEEYQCAWLDMYHRVFDRVSAVVGEQVWNFADFATSQGILRVGGNKKGIFTRDRKPKSAAFLLQKRWTGMNFGEKPQQGGKQ

SEQ ID NO: 3 - protein, 543 aa, Homo sapiens
MLLRSKPALPPPLMLLLLGPLGPLSPGALPRPAQAQDVVDLDFFTQEPLHLVSPSFLSVTIDANLATDPRFLILLGSPKLRTLARGLSPAYLRFGGTKTDFLIFDPKKESTFEERSYWQSQVNQDICKYGSIPPDVEEKLRLEWPYQEQLLLREHYQKKFKNSTYSRSSVDVLYTFANCSGLDLIFGLNALLRTADLQWNSSNAQLLLDYCSSKGYNISWELGNEPNSFLKKADIFINGSQLGEDFIQLHKLLRKSTFKNAKLYGPDVGQPRRKTAKMLKSFLKAGGEVIDSVTWHHYYLNGRTATKEDFLNPDVLDIFISSVQKVFQVVESTRPGKKVWLGETSSAYGGGAPLLSDTFAAGFMWLDKLGLSARMGIEVVMRQVFFGAGNYHLVDENFDPLPDYWLSLLFKKLVGTKVLMASVQGSKRRKLRVYLHCTNTDNPRYKEGDLTLYAINLHNVTKYLRLPYPFSNKQVDKYLLRPLGPHGLLSKSVQLNGLTLKMVDDQTLPPLMEKPLRPGSSLGLPAFSYSFFVIRNAKVAACI

SEQ ID NO: 4 - protein, 463 aa, Burkholderia pseudomallei
MLAACGGGGGADAAAAAPQQPPPAGPSSSANVAMTLPADAPRIARDFAGLSIEKAALSYPLLSGENGNMVGLFNRLGAGVLRIGGNSSDASGWQRTGPDETSGVITPAAVDRLASFVQACRWRVIYGLNFVGNDPATIADEAAYAAQALGVQLAGFEIGNEPDLYAQHGLAPNANTYPGEVSRWTTFANAIRAAVPDAVFTGPATAWNYQRYTVPFASDAAGLVSLLTQHHYRNPDSATIEAMLSPDPSLAPMLQALQGAASARGIGFRLAETNSYWGGGKPGVSDAHASALWVINFLFAVAQGGASGVNLHTGGGASYSAIKTNKTAGTVAAIGPEYYGIYLENQAAGGRLMQTRVDSAGTTLFAHAVAADGGGVRLILVNTDANSGYDVAVDCSSVPNARAGIVTTLGGPSLGSLTGTQIDGATFALDGSGAPQGGRPVACVNGVLGVHVASASALLVDFA

SEQ ID NO: 5 - protein, 475 aa, Acidobacterium capsulatum
MAFARGGLAQTASQTTSSPVRVGLSVDASALGHTIPPDYTGLSYEQAQMANPNYFSGANTQLAGFLRTLGRQGVLRIGGNTSEYTFWNRHAKPTAADEHLAAGPDKGHHAAAREVITPEAVNNLSEFLDKTGWKLIYGLNLGKGTPENAADEAAYVMETIGADRLLAFQLGNEPDLFYRNGIRPASYDFAAYAGDWQRFFTAIRKRVPNAPFAGPDTAYNTKWLVPFADKFKHDVKFISSHYYAEGPPTDPSMTIERLMKPNPRLLGETAGLKQVEADTGLPFRLTETNSCYQGGKQGVSDTFAAALWAGDLMYQQAAAGSTGINFHGGGYGWYTPVAGTPEDGFIARPEYYGMLLFAQAGAGQLLGAKLTDNSAAPLLTAYALRGTDGRTRIALFNKNLDADVEVAISGVASPSGTVLRLEAPRADDTTDVTFGGAPVGASGSWSPLVQEYVPGHSGQFVLHMRKASGALLEFA